European Patent Application EP 4 464 723 A1, published November 20, 2024. Title: Fusion Protein Comprising Modified Anti-VEGFR2(KDR) Antibody and Use Thereof. Applicant: Pharmabcine Inc. The sequence listing filed with the application follows.

SEQUENCE LISTING (36 sequences)

SEQ ID NO: 1 - protein, 8 aa, synthetic construct
  REGION 1..8: note = Heavy-chain CDR1
GYTFSSYW

SEQ ID NO: 2 - protein, 8 aa, synthetic construct
  REGION 1..8: note = Heavy-chain CDR2
INPGNGHT

SEQ ID NO: 3 - protein, 14 aa, synthetic construct
  REGION 1..14: note = Heavy-chain CDR3
ARHWGPSLTSPFDY

SEQ ID NO: 4 - protein, 6 aa, synthetic construct
  REGION 1..6: note = Light-chain CDR1
NLGDVN

SEQ ID NO: 5 - skipped

SEQ ID NO: 6 - protein, 10 aa, synthetic construct
  REGION 1..10: note = Light-chain CDR3
QAPTNNDPYT

SEQ ID NO: 7 - DNA, 363 bp, synthetic construct
  misc_feature 1..363: note = VH
  source 1..363: mol_type = other DNA
gaggtgcagctggtggaatccggcggaggactggtgcagcctggcggctccctgagactgtcttgcgccgcctccggatacaccttcagcagctactggatgagctgggtgcgacaggcccctggcaagggcctcgaatgggtgtcagagattaatcctggcaacggtcatactaactacaacgagaagttcaagtcacggttcaccatctccagagacaagtccaagaacaccctgtacctgcagatgaactccctgcgggccgaggacaccgccgtgtactactgcgccagacattggggcccgagtcttacttctccctttgactactggggccagggcaccctggtgacagtgtcctcc

SEQ ID NO: 8 - protein, 121 aa, synthetic construct
  REGION 1..121: note = VH
EVQLVESGGGLVQPGGSLRLSCAASGYTFSSYWMSWVRQAPGKGLEWVSEINPGNGHTNYNEKFKSRFTISRDKSKNTLYLQMNSLRAEDTAVYYCARHWGPSLTSPFDYWGQGTLVTVSS

SEQ ID NO: 9 - DNA, 330 bp, synthetic construct
  misc_feature 1..330: note = VL
  source 1..330: mol_type = other DNA
gacatccagatgacccagtctccatcctccctgtctgcatctgtaggagacagagtcaccatcacttgccgggcagataaccttggagatgtaaatgtacactggtatcagcagaaaccagggaaagcccctaagctcctgatctattatgatgccgaccggccctcaggggtcccatcaaggttcagtggcagtaattctgggaatgatgccactctcaccatcagcagtctgcaacctgaagattttgcaacttactactgtcaagcaccaacaaacaacgatccttataccttcggccagggcaccaaggtggaaatcaagcggacc

SEQ ID NO: 10 - protein, 110 aa, synthetic construct
  REGION 1..110: note = VL
DIQMTQSPSSLSASVGDRVTITCRADNLGDVNVHWYQQKPGKAPKLLIYYDADRPSGVPSRFSGSNSGNDATLTISSLQPEDFATYYCQAPTNNDPYTFGQGTKVEIKRT

SEQ ID NO: 11 - DNA, 990 bp, synthetic construct
  misc_feature 1..990: note = Heavy-chain Constant Region
  source 1..990: mol_type = other DNA
gctagcaccaagggcccatcggtcttccccctggcaccctcctccaagagcacctctgggggcacagcggccctgggctgcctggtcaaggactacttccccgaaccggtgacggtgtcgtggaactcaggcgccctgaccagcggcgtgcacaccttcccggctgtcctacagtcctcaggactctactccctcagcagcgtggtgaccgtgccctccagcagcttgggcacccagacctacatctgcaacgtgaatcacaagcccagcaacaccaaggtggacaagaaagttgagcccaaatcttgtgacaaaactcacacatgcccaccgtgcccagcacctgaactcctggggggaccgtcagtcttcctcttccccccaaaacccaaggacaccctcatgatctcccggacccctgaggtcacatgcgtggtggtggacgtgagccacgaagaccctgaggtcaagttcaactggtacgtggacggcgtggaggtgcataatgccaagacaaagccgcgggaggagcagtacaacagcacgtaccgtgtggtcagcgtcctcaccgtcctgcaccaggactggctgaatggcaaggagtacaagtgcaaggtctccaacaaagccctcccagcccccatcgagaaaaccatctccaaagccaaagggcagccccgagaaccacaggtgtacaccctgcccccatcccgggaggagatgaccaagaaccaggtcagcctgacctgcctggtcaaaggcttctatcccagcgacatcgccgtggagtgggagagcaatgggcagccggagaacaactacaagaccacgcctcccgtgctggactccgacggctccttcttcctctacagcaagctcaccgtggacaagagcaggtggcagcaggggaacgtcttctcatgctccgtgatgcatgaggctctgcacaaccactacacgcagaagagcctctccctgtctcccggggca

SEQ ID NO: 12 - protein, 330 aa, synthetic construct
  REGION 1..330: note = Heavy-chain Constant Region
ASTKGPSVFPLAPSSKSTSGGTAALGCLVKDYFPEPVTVSWNSGALTSGVHTFPAVLQSSGLYSLSSVVTVPSSSLGTQTYICNVNHKPSNTKVDKKVEPKSCDKTHTCPPCPAPELLGGPSVFLFPPKPKDTLMISRTPEVTCVVVDVSHEDPEVKFNWYVDGVEVHNAKTKPREEQYNSTYRVVSVLTVLHQDWLNGKEYKCKVSNKALPAPIEKTISKAKGQPREPQVYTLPPSREEMTKNQVSLTCLVKGFYPSDIAVEWESNGQPENNYKTTPPVLDSDGSFFLYSKLTVDKSRWQQGNVFSCSVMHEALHNHYTQKSLSLSPGK

SEQ ID NO: 13 - DNA, 318 bp, synthetic construct
  misc_feature 1..318: note = Light-chain Constant Region
  source 1..318: mol_type = other DNA
acggtggctgcaccatctgtcttcatcttcccgccatctgatgagcagttgaaatctggaactgcctctgttgtgtgcctgctgaataacttctatcccagagaggccaaagtacagtggaaggtggataacgccctccaatcgggtaactcccaggagagtgtcacagagcaggacagcaaggacagcacctacagcctcagcagcaccctgacgctgagcaaagcagactacgagaaacacaaagtctacgcctgcgaagtcacccatcagggcctgagctcgcccgtcacaaagagcttcaacaggggagagtgt

SEQ ID NO: 14 - protein, 106 aa, synthetic construct
  REGION 1..106: note = Light-chain Constant Region
TVAAPSVFIFPPSDEQLKSGTASVVCLLNNFYPREAKVQWKVDNALQSGNSQESVTEQDSKDSTYSLSSTLTLSKADYEKHKVYACEVTHQGLSSPVTKSFNRGEC

SEQ ID NO: 15 - DNA, 60 bp, synthetic construct
  misc_feature 1..60: note = Linker
  source 1..60: mol_type = other DNA
ggtggcggaggatctggcggtggtggttctggcggaggcggaagtggcggtggcggatct

SEQ ID NO: 16 - protein, 20 aa, synthetic construct
  REGION 1..20: note = Linker
GGGGSGGGGSGGGGSGGGGS

SEQ ID NO: 17 - DNA, 231 bp, synthetic construct
  misc_feature 1..231: note = Notch1
  source 1..231: mol_type = other DNA
gacgtggacgagtgttctctgggcgccaatccttgtgaacacgccggcaagtgtatcaacaccctgggcagcttcgagtgccagtgtctgcagggctataccggacctagatgcgagatcgatgtgaacgagtgtgtgtctaacccctgccagaacgacgccacctgtctggatcagatcggcgagttccagtgcatctgcatgcctggatatgagggcgtgcactgtgaa

SEQ ID NO: 18 - protein, 77 aa, synthetic construct
  REGION 1..77: note = Notch1
DVDECSLGANPCEHAGKCINTLGSFECQCLQGYTGPRCEIDVNECVSNPCQNDATCLDQIGEFQCICMPGYEGVHCE

SEQ ID NO: 19 - DNA, 363 bp, synthetic construct; identical to SEQ ID NO: 7
  misc_feature 1..363: note = VH
  source 1..363: mol_type = other DNA

SEQ ID NO: 20 - protein, 121 aa, synthetic construct; identical to SEQ ID NO: 8
  REGION 1..121: note = VH

SEQ ID NO: 21 - DNA, 330 bp, synthetic construct
  misc_feature 1..330: note = VL
  source 1..330: mol_type = other DNA
gacatccagatgacccagtctccatcctccctgtctgcatctgtaggagacagagtcaccatcacttgccgggcagataaccttggagatgtaaatgtacactggtatcagcagaaaccagggaaagcccctaagctcctgatctattatgatgccgaccggccctcaggggtcccatcaaggttcagtggcagtaattctgggaatgatgccactctcaccatcagcagtctgcaacctgaagattttgcaacttactactgtcaagcgcccacaagaatagcgccttataccttcggccagggcaccaaggtggaaatcaagcggacc

SEQ ID NO: 22 - protein, 110 aa, synthetic construct
  REGION 1..110: note = VL
DIQMTQSPSSLSASVGDRVTITCRADNLGDVNVHWYQQKPGKAPKLLIYYDADRPSGVPSRFSGSNSGNDATLTISSLQPEDFATYYCQAPTRIAPYTFGQGTKVEIKRT

SEQ ID NO: 23 - DNA, 363 bp, synthetic construct
  misc_feature 1..363: note = VH
  source 1..363: mol_type = other DNA
gaggtgcagctggtggaatccggcggaggactggtgcagcctggcggctccctgagactgtcttgcgccgcctccggatacaccttcagcagctactggatgagctgggtgcgacaggcccctggcaagggcctcgaatgggtgtcagagattaatcctggcaacggtcatactaactacaacgagaagttcaagtcacggttcaccatctccagagacaagtccaagaacaccctgtacctgcagatgaactccctgcgggccgaggacaccgccgtgtactactgcgccagaagctaccgcccgagtcttacttctccctttgatttctggggccagggcaccctggtgacagtgtcctcc

SEQ ID NO: 24 - protein, 121 aa, synthetic construct
  REGION 1..121: note = VH
EVQLVESGGGLVQPGGSLRLSCAASGYTFSSYWMSWVRQAPGKGLEWVSEINPGNGHTNYNEKFKSRFTISRDKSKNTLYLQMNSLRAEDTAVYYCARSYRPSLTSPFDFWGQGTLVTVSS

SEQ ID NO: 25 - DNA, 330 bp, synthetic construct
  misc_feature 1..330: note = VL
  source 1..330: mol_type = other DNA
gacatccagatgacccagtctccatcctccctgtctgcatctgtaggagacagagtcaccatcacttgccgggcagataaccttggagatgtaaatgtacactggtatcagcagaaaccagggaaagcccctaagctcctgatctattatgatgccgaccggccctcaggggtcccatcaaggttcagtggcagtaattctgggaatgatgccactctcaccatcagcagtctgcaacctgaagattttgcaacttactactgtcaagcgccaaccaccaacgagccttataccttcggccagggcaccaaggtggaaatcaagcggacc

SEQ ID NO: 26 - protein, 110 aa, synthetic construct
  REGION 1..110: note = VL
DIQMTQSPSSLSASVGDRVTITCRADNLGDVNVHWYQQKPGKAPKLLIYYDADRPSGVPSRFSGSNSGNDATLTISSLQPEDFATYYCQAPTTNEPYTFGQGTKVEIKRT

SEQ ID NO: 27 - DNA, 363 bp, synthetic construct; identical to SEQ ID NO: 7
  misc_feature 1..363: note = VH
  source 1..363: mol_type = other DNA

SEQ ID NO: 28 - protein, 121 aa, synthetic construct; identical to SEQ ID NO: 8
  REGION 1..121: note = VH

SEQ ID NO: 29 - DNA, 330 bp, synthetic construct
  misc_feature 1..330: note = VL
  source 1..330: mol_type = other DNA
gacatccagatgacccagtctccatcctccctgtctgcatctgtaggagacagagtcaccatcacttgccgggcagataaccttggagatgtaaatgtacactggtatcagcagaaaccagggaaagcccctaagctcctgatctattatgatgccgaccggccctcaggggtcccatcaaggttcagtggcagtaattctgggaatgatgccactctcaccatcagcagtctgcaacctgaagattttgcaacttactactgtcaagcaccaaccacgcatctgccttataccttcggccagggtaccaaggtggaaatcaagcggacc

SEQ ID NO: 30 - protein, 110 aa, synthetic construct
  REGION 1..110: note = VL
DIQMTQSPSSLSASVGDRVTITCRADNLGDVNVHWYQQKPGKAPKLLIYYDADRPSGVPSRFSGSNSGNDATLTISSLQPEDFATYYCQAPTTHLPYTFGQGTKVEIKRT

SEQ ID NO: 31 - DNA, 363 bp, synthetic construct; identical to SEQ ID NO: 7
  misc_feature 1..363: note = VH
  source 1..363: mol_type = other DNA

SEQ ID NO: 32 - protein, 121 aa, synthetic construct; identical to SEQ ID NO: 8
  REGION 1..121: note = VH

SEQ ID NO: 33 - DNA, 330 bp, synthetic construct
  misc_feature 1..330: note = VL
  source 1..330: mol_type = other DNA
gacatccagatgacccagtctccatcctccctgtctgcatctgtaggagacagagtcaccatcacttgccgggcagataaccttggagatgtaaatgtacactggtatcagcagaaaccagggaaagcccctaagctcctgatctattatgatgccgaccggccctcaggggtcccatcaaggttcagtggcagtaattctgggaatgatgccactctcaccatcagcagtctgcaacctgaagattttgcaacttactactgtcaagcgccaaccaaaaacgtcccttataccttcggccagggcaccaaggtggaaatcaagcggacc

SEQ ID NO: 34 - protein, 110 aa, synthetic construct
  REGION 1..110: note = VL
DIQMTQSPSSLSASVGDRVTITCRADNLGDVNVHWYQQKPGKAPKLLIYYDADRPSGVPSRFSGSNSGNDATLTISSLQPEDFATYYCQAPTKNVPYTFGQGTKVEIKRT

SEQ ID NO: 35 - protein, 116 aa, synthetic construct
  REGION 1..116: note = Heavy-chain
QMQLVQSGAEVKKPGASVKLSCKASGYTFSSYWMHWVRQAPGQRLEWMGEINPGNGHTNYNEKFKSRVTITVDKSASTAYMELSSLRSEDTAVYYCAKIWGPSLTSPFDYWGQGTL

SEQ ID NO: 36 - protein, 198 aa, synthetic construct
  REGION 1..198: note = Light-chain
DVDECSLGANPCEHAGKCINTLGSFECQCLQGYTGPRCEIDVNECVSNPCQNDATCLDQIGEFQCICMPGYEGVHCESGGGGSGGGGSGSNFMLTQPPSVSVSPGKTARITCRGDNLGDVNVHWYQQRPGQAPVLVMYYDADRPSGIPERFSGSNSGNTATLTISGVEAGDEADYYCQVWDRTSEYVFGTGTKVTVLG